European Patent Application EP 4 155 393 A1, published March 29, 2023. Title: ATTENUATED VARIANT OF THE RIFT VALLEY FEVER VIRUS, COMPOSITION COMPRISING SAME, AND USES THEREOF. Applicant: CONSEJO SUPERIOR DE INVESTIGACIONES CIENTÍFICAS (CSIC). Application EP21818246. The sequence listing filed with the application follows.

SEQUENCE LISTING (57 sequences)

SEQ ID NO: 1 - DNA, 6404 bp, Artificial Sequence
  FMH-P8 RVF virus L segment
  gene 19..6297: /note="FMH-P8 RVF virus L-segment open reading frame"
acacaaaggcgcccaatcatggattctatattatcaaaacagctggttgacaagactggttttgttagagtgccaatcaagcattatgactgtacaatgctaactctggcactcccaacatttgatgtctccaagatggtagatagaattaccatagacttcaatttagacgacatacaaggagcatctgaaataggttcaactttgctaccctctatgtcgatagatgtggaagatatggccaattttgttcacgatttcacctttggccacttagctgacaagactgacagactcttaatgcgtgagtttcccacgatgaatgacgggtttgatcatctgagccctgacatgattatcaaaactacatctggcatgtataacatcgttgagtttaccacctttaggggggatgaaagaggtgcattccaggctgccatgactaaactcgctaagtatgaggttccttgtgagaacagatctcagggcaggactgttgttctttatgttgttagcgcctaccggcatggtgtttggtctaatttggagctagaggactctgaagcagaggagatggtatataggtacagacttgcccttagtgtgatggatgagctaaggaccttgttcccagaactgtcatccacagatgaggaactaggaaagactgagagagagttgctagccatggtctcctccatccaaataaattggtcagtcacagaatctgtgtttcctccctttagcagagaaatgtttgacaggttcagatcttctcctcccgattcagagtacatcacgaggatagtgagcagatgcctcataaattctcaagagaaactcatcaataattccttctttgctgaagggaatgataaagttttgagattttcaaaaaacgctgaggagtgttccttggcaatagagagagctttaaatcagtatagggcagaagacaaccttagggacctcaatgaccacaagtctactattcagctgcccccctggctgtcctatcacgatgccgatggcaaagatctgtgccctcttcagggattagatgtgagaggagaccatcccatgtgcaacctgtggagagaagtggttacctctgcaaatttagaggagattgagaggatgtacgatgatgcagcggcagaacttgagtttgccctttcaggggtgaaggacaggccagatgaaagaaacagataccatagagtccatctgaatatggactcagatgatagtgtctacatagctgctttaggggttaatggaaagaagcataaagcagacacattagtgcaacaaatgagagacaggagcaaacagcccttctctccagatcatgatgtggatcacatatctgaatttctctctgcatgctctagtgacttgtgggcaacagatgaggacctatacaaccctctctcttgtgataaagagcttagattggcagctcagagaattcatcagccatccttatcagaaaggggcttcaatgagattataacagagcactacagatttatgggaagtaggataggatcatggtgccaaatggtcagtttaataggagctgagctatcagcttctgtaaagcaacatgttaagcctaactattttgtgattaaacgactactaggttctgggattttcttgctgatcaagcctacttccagcaaaagccatatattcgtgtcttttgcaattaagcgctcttgctgggcctttgatctctccacttccagggttttcaaaccctacatagatgccggggatctgttagttactgactttgtttcttacaaactaagtaagcttaccaacctctgcaagtgcgtttcgttaatggaatcctccttctcattttgggcagaggcatttgggattccaagctggaactttgttagtgacttgttcaggtcttcagactctgcagcaatggatgcctcatacatgggcaaactctctttattaacccttttggaagacaaagcaacaactgaagagttacagactattgcaagatatataatcatggagggctttgtctcgcccccagaaatcccaaaacctcacaagatgacctctaagtttcccaaggttctcaggtcagagctgcaggtttacttattaaactgcttatgcagaactatccagagaatagcaggtgagccctttattcttaagaagaaggatgggtctatatcctggggtggcatgtttaatcctttttcagggcgtccactgcttgatatgcaaccactcatcagctgttgttacaatggttactttaaaaacaaagaagaagagactgagccttcctccctttctgggatgtataagaaaattatagaacttgagcaccttagaccacagtcagatgccttcttgggttataaagatccagaactacctagaatgcatgagttcagtgtttcctacttgaaggaggcttgcaatcatgctaagctggtcttaaggagtctctatggacagaatttcatggagcaaatagacaaccaaattattcgagagctcagtgggttgactctagaaagattagccacacttaaggccacaagcaactttaatgagaattggtatgtctataaggatgtggcagacaagaactacacaagggataaattattagtgaagatgtcaaaatatgcttctgagggaaagagcctagctatccagaagtttgaggattgcatgaggcagatagagtcacaaggatgtatgcatatttgtttgtttaagaaacaacagcatggaagtctgagagagatctatgtgatgggtgcagaggaaagaattgttcaatcggtggtggagacaatagccaggtctatagggaagttctttgcttctgataccctctgtaacccccccaataaggtgaaaattcctgagacacatggcattagggctcggaagcaatgtaaggggcctgtgtggacttgtgcaacatcagatgatgcaaggaagtggaaccaaggccattttgttacaaagtttgccctcatgctatgtgagttcacctctcctaagtggtggccattgatcattaggggatgttcaatgtttaccaggaaaaggatgatgatgaatttgaattatcttaagatcctggatggtcatcgagagcttgatgttagagatgactttgtgatggatctcttcaaagcttatcatggtgaggcagaagttccatgggcttttaagggtaaaacatatctggaaaccacaacagggatgatgcaggggatattgcattatacttcctcattattacacaccattcatcaagaatacatccggtccttgtcctttaaaatattcaacctgaaggttgctcctgagatgagcaaaagcctggtttgtgacatgatgcaaggatcagatgatagtagcatgctaatcagcttcccagctgatgacgagaaggttctcaccagatgcaaagtggccgcagccatatgcttccgaatgaagaaggagctgggagtgtaccttgccatctacccctcagagaagtccacagcaaacacagattttgtgatggagtacaattctgaattttatttccacacccagcatgttagaccgacgatcaggtggattgcagcatgttgcagcctgccagaagtggaaacactagtagcccgccaggaagaggcctctaatctaatgacttcagttactgaggggggtgggtcattctccttagctgcaatgattcagcaagctcagtgcactctccattacatgctaatgggcatgggagtgtctgagctattcttagagtataagaaggcagtgctgaagtggaatgaccctggtctgggtttcttcctgcttgacaatccttatgcgtgcgggttgggaggttttagatttaatctcttcaaaaccatcaccagaactgatttgcagaagctatatgctttcttcatgaagaaggttaagggctcagctgctagggactgggcagatgaggatgttaccatcccagaaacgtgtagcgtgagcccaggtggcgctctaattcttagctcctctctaaagtggggatctaggaagaagtttcagaaactaagagaccgtttgaacataccagagaactggattgagctaataaatgagaatccagaggtgctctatcgagctcccagaacaggcccagaaatattgttgcgcattgcagagaaagtccatagccctggtgttgtgtcatcattgtcttctggcaatgcagtctgtaaagtcatggcctcagctgtatacttcttatcagcaacaatttttgaagacactggacgccctgagttcaacttcttagaggattccaagtacagcttgctacaaaagatggccgcatattctggctttcatggtttcaatgatatggagccagaagatatattattcctattcccgaacattgaggaattagaatcactggattctatagtttacaacaagggagaaatagacatcatcccaagagttaatatcagggatgcaacccaaaccagggtcactatctttaatgagcagaagaccctccgaacatctccagagaagttggtgtcagacaagtggttcgggactcagaagagtaggataggcaaaacaactttcctggctgaatgggagaagctaaagaaaattgtgaagtggttggaagacactccagaagcaactctagctcacactccactgaataaccatattcaggttaggaatttctttgctagaatggaaagcaagcctagaacggttagaataacaggagctcctgtaaagaagaggtcaggggttagcaagatagctatggttatccgtgacaatttctcccggatgggccatcttagaggtgtagaagacttcgctggcttcactcgtagtgtgtcagctgaaatcctcaagcactttctgttctgcatactacagggtccatacagtgagagctataaactacagctaatctacagagtcctaagctcagtatcaaacgttgagataaaggaatcggatggtaagacaaaaaccaatttgattgggatccttcagagatttctagatggtgatcacgttgtccctataattgaagagatgggagccggaacagtgggtggattcatcaagagacaacagtctaaagttgtgcaaaataaggtggtctattatggagttgggatctggagaggctttatggatggatatcaggtccatcttgagatagaaaatgacataggacagcccccaaggcttaggaatgtcacaactaactgtcagagcagcccatgggatctgagtgtcccaataaggcagtgggcagaagacatgggggtcacaaacaaccaggattattcctctaaatctagcagaggagctagatattggatgcattcatttaggatgcaaggacccagcaagccatttggatgcccagtttatattattaagggtgacatgtcagatgttatcagactgagaaaagaggaggtggagatgaaagtacggggctctactctcaacttgtacactaagcaccattctcatcaagacttacacattttatcttacactgcatcagacaatgatctcagtccaggcattttcaagtcaatatcagatgagggagtggctcaagccctgcagttatttgagagggagccaagcaactgctgggtgagatgtgagtctgtagctccaaaattcatatcagccatccttgagatatgtgaggggaagagacagataaaaggaatcaacagaaccagactctcagagattgtgagaatttgttctgaatcttccctaagatcaaaggtcggatctatgttctcatttgtcgccaatgttgaggaggcccatgatgttgattatgatgcgttaatggatctaatgatagaagatgctaagaacaatgcattcagtcatgttgtcgattgcatagagttggatgttaatggtccttacgagatggagtcttttgatacatctgatgtcaacctctttgggccagcccattacaaggacatcagttcattatctatgattgctcatcccttaatggataagtttgttgattatgccatttccaagatggggagagcctcagttagaaaagttctagagacaggtcggtgctctagcaaagactatgatttatcaaaggttctcttcagaactctacagagaccagaaaagagcattaggatagatgatctggagttatatgaggagacagatgtggcggatgacatgctaggctaagaccaataagcaaagtcaggcttagatttagggatactacgctagtattggaatccatgtgggttctgatactagcatagtgctacaatattgggcggtctttgtgt

SEQ ID NO: 2 - DNA, 3885 bp, Artificial Sequence
  FMH-P8 RVF virus M segment
  gene 21..3614: /note="FMH-P8 RFV virus gene encoding M (poly)protein"
acacaaagacggtgcattaaatgtatgttttactaacaattctgatcacggttctggtgtgtgaagcggttattagagtgtctctaagctccacaaaagaagagacctgttttggtgactccaccaacccagagatgattgaaggagcttgggattcactcagagaggaggagatgccagaggagctctcctgttctatatcaggcataagggaggttaagacctcaagccaggagttatacagggcattaaaagccatcattgctgctgatggcttgaacaacatcacctgccatggtaaggatcctgaggacaagatttctctcataaagggtcctccttacaaaaagcgggtggggatagttcggtgtaaaagacgaagagatgctaagcaaatagggagagaaaccatggcagggattgcaatgacagtccttccagccttagcagtttttgctttggcacctgttgtttttgctgaagacccccatctcaggaacagaccagggaaggggcacaactacattgacgggatgactcaggaggatgccacatgcaaacctgtgacatatgctggggcatgtagcagttttgatgtcttgcttgaaaaggggaaatttccccttttccagtcgtatgctcatcataaaactctactggaagcagttcacgacactatcattgcaaaggctgatccacctagctgtgaccttcaaagtgctcatgggaatccctgcatgaaagagaaactcgtgatgaagacacactgtccaaatgactaccagtcagctcattacctcaacaatgacgggaaagtggcttcagtcaagtgccctcctaagtatgagctcactgaggactgcaacttttgtaggcagatgacaggtgctagcctgaagaaagggtcttatcctctccaagacttattttgtcagtcaagtgaggatgatggatcaaaattaaaaacaaaaatgaaaggggtctgcgaagtgggggttcaagcactcaaaaagtgtaatggccaactcagcactgcacatgaggttgtgccctttgcagtgtttaagaactcaaagaaagtttatcttgataagcttgacctcaaaactgaggagaatctgctaccagactcatttgtctgcttcgagcataagggacagtataaaggaacaatggactctggtcagactaagagggagctcaaaagctctgatatctctcagtgccccaagattggaggacatggtagtaaaaagtgcactggggacgcagcattttgctctgcttatgagtgcactactcagtacgccaatgtctactgttcacatgctaatggatcagggattgtgcagatacaagtatcaggggtctggaagaagcctttatgtgtagggtatgagagagtggttgtgaagagagaactctctgccaagcccatccagagagttgagccctgcacaacttgtataaccaaatgtgggcctcatggattggttgtccgatcaacagggttcaagatatcatctgcagttgcttgtgctagcggagtttgcgtcacaggatcgcagagtccttctaccgagattacactcaagtatccagggatatcccagtcctctgggggggacataggggtttacatggcacatgatgatcagtcagttagctccaaaatagtagctcactgccccccccaggacccgtgcttagtgcatggctgcatagtgtgtgctcatggcctaataaattaccagtgtcacactactctcagtgcctttattgttgtgtttgtattcagttctattgcaataacttgtttagctattctttatagggtgctcaagtgcctaaagattgccccaaggaaggttctaaatccactaatgtggattacagccttcatcagatgggtgtataagaagatggttgctagagtggcagacaatattaatcaagtgaacagggaaataggatggatggaagggggtcagttggttctagggaaccctgcccctattcctcgtcatgccccaatcccacgttatagcacatacctaatgctactattgattgtctcatatgcatcagcatgttcagaactgattcaggcaagctccagaatcaccacttgctccacagagggtgttaacaccaagtgtagactgtctggcacagcattgatcagggcagggtcagttggggcagaggcttgtttaatgttgaagggggtcaaggaagatcaaaccaaattcttgaagataaaaactgtctcaagtgagctatcgtgcagggagggccagagctattggactgggtcctttagtcccaaatgtctgagctcaaggagatgccatcttgttggagaatgtcatgtgaataggtgtctgtcttggagggacaatgaaacttcagcagagttttcatttgttggggaaagcacgaccatgcgagagaataagtgttttgagcagtgtggaggatgggggtgtgggtgcttcaatgtgaacccatcttgcttatttgtgcacacgtacctgcagtcagttagaaaagaggcccttagagtttttaactgtatcgactgggtgcataaactcagtctagagatcacagactttgatggctctgtttcaacaatagacttgggagcatcatctagccgtttcacaaactggggttcagttagcctctcactggacgcagagggtatttcaggctcaaatagcttttctttcattgagagcccaggcaaagggtatgcaattgttgatgagccattctcagaaattcctcggcaagggttcttgggggagatcaggtgtaattcagagtcctcagtcctgagtgctcatgaatcatgccttagggtaccaaaccttatctcatacaagcccatgatagatcaattggagtgcacaacaaatctgattgatccttttgttgtctttgagaggggttctctgccacagacaaggaatgaaaaaacctttgcagcttcaaaaggaaataggggtgttcaagctttctctaagggctctgtacaagctgatctaactctgatgtttgacaattttgaggtggactttgtgggagcagccgtatcttgtgatgccgccttcttaaacttgacaggttgctattcttgcaatgcgggagccagggtctgcctgtctatcacatccacaggaactggaactctctctgcccacaataaggatgggtctctgcacatagttcttccatcagagaatggaacaaaagatcagtgtcagatactacacttcactatacctgaagtagaggaggagtttatgtactcttgtgatggagatgagcggcctctgttggtgaaagggactctgatagttattgatccatttgatgataggcgggaagcagggggggaatcaacagttgtgaatccaaaatctggatcttggaatttctttgactggttttctggactcatgagttggtttggagggcctcttaaaactatactcctcatttgcctgtatgttgcattatcaattgggctctttttcctccttatatatcttggaaaaacaggcctctctaaaatgtggcttgctgctactaagaaggcctcatagatcagtacgtgtagaagcaatatgtagaaacaagtggacataagcaaacctaattatgtaaatattgtacagataggtcaaattattgggatatccaagcttagatgcttatgcaatattacttttgatgtaagcttagttgtaatttggggtggtggggtgaggcagcagcagtctcaagtgcttgtgaatattctagttggcgtgaatgtcttttgccagattagctgggaattaaactaactctttgaagttgcaccggtctttgtgt

SEQ ID NO: 3 - DNA, 1691 bp, Artificial Sequence
  FMH-P8 RVF virus S segment
  gene 35..832: /note="FMH-P8 RVF virus gene encoding NSs protein"
  gene 916..1653: /note="FMH-P8 RVFV gene encoding N protein (complementary)"
acacaaagaccccctagtgcttatcaagtgtatcatggattactttcctgtgatatctgttgatttgcagagtggtcgtcgtgttgtgtcagtggagtacattagaggtgatggtcctcccagaataccttattctatggttgggccctgttgtgtctttctcatgcaccatcgtcctagtcacgagattcgcttgcgattctctgatttctacaatgtcggagaattcccataccgagtcggacttggagactttgtatcaaacgttgcacctccactagcaaagccttttcagagacttattgatctaataggccatatgactcttagtgatttcacaaggttccccaatctgaaagaagccatatcctggcctcttggagaaccctccctggctttctttgacctaagctccaccagagtgcataggtctgatgatattagaagggaccagattgctactctagcaatgaggagctgcaagattaccaatgatctggaggactcctttgttggcttacacaggatgatagtgaccgaggctatcctcagagggattgacttgtgcctgttgccaggctttgatctcatgtatgaagttgctcacgttcagtgtgttcggctcctgcaggcagcaagagaggatatttctaatgctgtagttccaaactcagctctcattgctcttatggaggagagcttgatgctgcgctcatcactccctagcatgatggggagaaacaactgggttccagttgttcctccaatcccagatgttgagatagaatcagaggaagagagtgatgacgatggatttgttgaggttgattagagattaaggctgccccaccccccacccccaatcccgaccgtaaccccaaccacctccttttccccaaacccctgggcagccacttaggctgctgtcttgtacgcctgagcagctgccataacagctgctgacggcttcccattggaatccacaagcccaaaagctttcaagaattctctcctcttctcatggcttataaagttgctattcactgctgcattcattggctgcgtgaacgttgcggcaacctcctcctttgttctacctcggaggtttgggttgatgacccgggagaactgcagcagatacagagagtgagcatccaatattgcccttagatagtcttctggtagagaagggtccaccatgccagcaaagctggggtgcatcatatgccttgggtatgcaggggataggccatccatggtggtcccagtgacaggaagccactcactcaagacgaccaaagcctggcaagtccagccagccagggcagcagcaactcgtgatagagtcaactcatcccgggaaggattcccctcctttagcttatacttgttgatgagagcctccacagttgctttgccttctttcgacattttcatcatcatcctccggggcttgttgccacgagtcagagccagaacaatcattttcttggcatccttctcccagccagccccaccatactgctttaagagttcgataaccctacgggcatcaaatccttgataagcaaactctcggacccactgttcaatctcattgcggtccactgcttgagcagcaaactggatcgcaagctcttgataattgtccattattgtaatagtgtttgtatctctagggagctttgtgt

SEQ ID NO: 4 - protein, 2092 aa, Artificial Sequence
  FMH-P8 RVFV L protein
  MUTAGEN 100: Thr
  MUTAGEN 375: Tyr
  MUTAGEN 924: Ser
  MUTAGEN 1050: Val
  MUTAGEN 1303: Thr
  MUTAGEN 1629: Phe
  MUTAGEN 2071: Lys
MDSILSKQLVDKTGFVRVPIKHYDCTMLTLALPTFDVSKMVDRITIDFNLDDIQGASEIGSTLLPSMSIDVEDMANFVHDFTFGHLADKTDRLLMREFPTMNDGFDHLSPDMIIKTTSGMYNIVEFTTFRGDERGAFQAAMTKLAKYEVPCENRSQGRTVVLYVVSAYRHGVWSNLELEDSEAEEMVYRYRLALSVMDELRTLFPELSSTDEELGKTERELLAMVSSIQINWSVTESVFPPFSREMFDRFRSSPPDSEYITRIVSRCLINSQEKLINNSFFAEGNDKVLRFSKNAEECSLAIERALNQYRAEDNLRDLNDHKSTIQLPPWLSYHDADGKDLCPLQGLDVRGDHPMCNLWREVVTSANLEEIERMYDDAAAELEFALSGVKDRPDERNRYHRVHLNMDSDDSVYIAALGVNGKKHKADTLVQQMRDRSKQPFSPDHDVDHISEFLSACSSDLWATDEDLYNPLSCDKELRLAAQRIHQPSLSERGFNEIITEHYRFMGSRIGSWCQMVSLIGAELSASVKQHVKPNYFVIKRLLGSGIFLLIKPTSSKSHIFVSFAIKRSCWAFDLSTSRVFKPYIDAGDLLVTDFVSYKLSKLTNLCKCVSLMESSFSFWAEAFGIPSWNFVSDLFRSSDSAAMDASYMGKLSLLTLLEDKATTEELQTIARYIIMEGFVSPPEIPKPHKMTSKFPKVLRSELQVYLLNCLCRTIQRIAGEPFILKKKDGSISWGGMFNPFSGRPLLDMQPLISCCYNGYFKNKEEETEPSSLSGMYKKIIELEHLRPQSDAFLGYKDPELPRMHEFSVSYLKEACNHAKLVLRSLYGQNFMEQIDNQIIRELSGLTLERLATLKATSNFNENWYVYKDVADKNYTRDKLLVKMSKYASEGKSLAIQKFEDCMRQIESQGCMHICLFKKQQHGSLREIYVMGAEERIVQSVVETIARSIGKFFASDTLCNPPNKVKIPETHGIRARKQCKGPVWTCATSDDARKWNQGHFVTKFALMLCEFTSPKWWPLIIRGCSMFTRKRMMMNLNYLKILDGHRELDVRDDFVMDLFKAYHGEAEVPWAFKGKTYLETTTGMMQGILHYTSSLLHTIHQEYIRSLSFKIFNLKVAPEMSKSLVCDMMQGSDDSSMLISFPADDEKVLTRCKVAAAICFRMKKELGVYLAIYPSEKSTANTDFVMEYNSEFYFHTQHVRPTIRWIAACCSLPEVETLVARQEEASNLMTSVTEGGGSFSLAAMIQQAQCTLHYMLMGMGVSELFLEYKKAVLKWNDPGLGFFLLDNPYACGLGGFRFNLFKTITRTDLQKLYAFFMKKVKGSAARDWADEDVTIPETCSVSPGGALILSSSLKWGSRKKFQKLRDRLNIPENWIELINENPEVLYRAPRTGPEILLRIAEKVHSPGVVSSLSSGNAVCKVMASAVYFLSATIFEDTGRPEFNFLEDSKYSLLQKMAAYSGFHGFNDMEPEDILFLFPNIEELESLDSIVYNKGEIDIIPRVNIRDATQTRVTIFNEQKTLRTSPEKLVSDKWFGTQKSRIGKTTFLAEWEKLKKIVKWLEDTPEATLAHTPLNNHIQVRNFFARMESKPRTVRITGAPVKKRSGVSKIAMVIRDNFSRMGHLRGVEDFAGFTRSVSAEILKHFLFCILQGPYSESYKLQLIYRVLSSVSNVEIKESDGKTKTNLIGILQRFLDGDHVVPIIEEMGAGTVGGFIKRQQSKVVQNKVVYYGVGIWRGFMDGYQVHLEIENDIGQPPRLRNVTTNCQSSPWDLSVPIRQWAEDMGVTNNQDYSSKSSRGARYWMHSFRMQGPSKPFGCPVYIIKGDMSDVIRLRKEEVEMKVRGSTLNLYTKHHSHQDLHILSYTASDNDLSPGIFKSISDEGVAQALQLFEREPSNCWVRCESVAPKFISAILEICEGKRQIKGINRTRLSEIVRICSESSLRSKVGSMFSFVANVEEAHDVDYDALMDLMIEDAKNNAFSHVVDCIELDVNGPYEMESFDTSDVNLFGPAHYKDISSLSMIAHPLMDKFVDYAISKMGRASVRKVLETGRCSSKDYDLSKVLFRTLQRPEKSIRIDDLELYEETDVADDMLG

SEQ ID NO: 5 - protein, 1197 aa, Artificial Sequence
  FMH-P8 RVFV M (poly)protein
  MUTAGEN 26: Lys
  MUTAGEN 108: Tyr
  MUTAGEN 118: Lys
  MUTAGEN 210: Lys
  MUTAGEN 333: Asn
  MUTAGEN 427: Thr
  MUTAGEN 432: Val
  MUTAGEN 487: Gly
  MUTAGEN 540: Tyr
  MUTAGEN 582: Thr
  MUTAGEN 587: Ile
  MUTAGEN 950: Val
  MUTAGEN 1090: Ile
  MUTAGEN 1116: Val
  MUTAGEN 1182: Lys
MYVLLTILITVLVCEAVIRVSLSSTKEETCFGDSTNPEMIEGAWDSLREEEMPEELSCSISGIREVKTSSQELYRALKAIIAADGLNNITCHGKDPEDKISLIKGPPYKKRVGIVRCKRRRDAKQIGRETMAGIAMTVLPALAVFALAPVVFAEDPHLRNRPGKGHNYIDGMTQEDATCKPVTYAGACSSFDVLLEKGKFPLFQSYAHHKTLLEAVHDTIIAKADPPSCDLQSAHGNPCMKEKLVMKTHCPNDYQSAHYLNNDGKVASVKCPPKYELTEDCNFCRQMTGASLKKGSYPLQDLFCQSSEDDGSKLKTKMKGVCEVGVQALKKCNGQLSTAHEVVPFAVFKNSKKVYLDKLDLKTEENLLPDSFVCFEHKGQYKGTMDSGQTKRELKSSDISQCPKIGGHGSKKCTGDAAFCSAYECTTQYANVYCSHANGSGIVQIQVSGVWKKPLCVGYERVVVKRELSAKPIQRVEPCTTCITKCGPHGLVVRSTGFKISSAVACASGVCVTGSQSPSTEITLKYPGISQSSGGDIGVYMAHDDQSVSSKIVAHCPPQDPCLVHGCIVCAHGLINYQCHTTLSAFIVVFVFSSIAITCLAILYRVLKCLKIAPRKVLNPLMWITAFIRWVYKKMVARVADNINQVNREIGWMEGGQLVLGNPAPIPRHAPIPRYSTYLMLLLIVSYASACSELIQASSRITTCSTEGVNTKCRLSGTALIRAGSVGAEACLMLKGVKEDQTKFLKIKTVSSELSCREGQSYWTGSFSPKCLSSRRCHLVGECHVNRCLSWRDNETSAEFSFVGESTTMRENKCFEQCGGWGCGCFNVNPSCLFVHTYLQSVRKEALRVFNCIDWVHKLSLEITDFDGSVSTIDLGASSSRFTNWGSVSLSLDAEGISGSNSFSFIESPGKGYAIVDEPFSEIPRQGFLGEIRCNSESSVLSAHESCLRVPNLISYKPMIDQLECTTNLIDPFVVFERGSLPQTRNEKTFAASKGNRGVQAFSKGSVQADLTLMFDNFEVDFVGAAVSCDAAFLNLTGCYSCNAGARVCLSITSTGTGTLSAHNKDGSLHIVLPSENGTKDQCQILHFTIPEVEEEFMYSCDGDERPLLVKGTLIVIDPFDDRREAGGESTVVNPKSGSWNFFDWFSGLMSWFGGPLKTILLICLYVALSIGLFFLLIYLGKTGLSKMWLAATKKAS

SEQ ID NO: 6 - protein, 265 aa, Artificial Sequence
  FMH-P8 RVFV NSs protein
  MUTAGEN 52: Ile
  MUTAGEN 82: Leu
MDYFPVISVDLQSGRRVVSVEYIRGDGPPRIPYSMVGPCCVFLMHHRPSHEIRLRFSDFYNVGEFPYRVGLGDFVSNVAPPLAKPFQRLIDLIGHMTLSDFTRFPNLKEAISWPLGEPSLAFFDLSSTRVHRSDDIRRDQIATLAMRSCKITNDLEDSFVGLHRMIVTEAILRGIDLCLLPGFDLMYEVAHVQCVRLLQAAREDISNAVVPNSALIALMEESLMLRSSLPSMMGRNNWVPVVPPIPDVEIESEEESDDDGFVEVD

SEQ ID NO: 7 - protein, 245 aa, Artificial Sequence
  FMH-P8 RVFV N protein
MDNYQELAIQFAAQAVDRNEIEQWVREFAYQGFDARRVIELLKQYGGAGWEKDAKKMIVLALTRGNKPRRMMMKMSKEGKATVEALINKYKLKEGNPSRDELTLSRVAAALAGWTCQALVVLSEWLPVTGTTMDGLSPAYPRHMMHPSFAGMVDPSLPEDYLRAILDAHSLYLLQFSRVINPNLRGRTKEEVAATFTQPMNAAVNSNFISHEKRREFLKAFGLVDSNGKPSAAVMAAAQAYKTAA

SEQ ID NO: 8 - DNA, 30 bp, Artificial Sequence
  5’ end L segment primer
acacaaaggcgcccaatcatggattctata

SEQ ID NO: 9 - DNA, 17 bp, Artificial Sequence
  716F primer
cagtcacagaatctgtg

SEQ ID NO: 10 - DNA, 17 bp, Artificial Sequence
  L-F segment 1028ag primer
atggcaaagatctgtgc

SEQ ID NO: 11 - DNA, 20 bp, Artificial Sequence
  L-R 2300g primer
aagtaaccattgtaacaaca

SEQ ID NO: 12 - DNA, 23 bp, Artificial Sequence
  RdRp central-F primer
gctatccagaagtttgaggattg

SEQ ID NO: 13 - DNA, 23 bp, Artificial Sequence
  L-F segment primer
ttctttgcttctgataccctctg

SEQ ID NO: 14 - DNA, 23 bp, Artificial Sequence
  L-R segment primer
gttccacttccttgcatcatctg

SEQ ID NO: 15 - DNA, 23 bp, Artificial Sequence
  Central-R RdRp primer
ctgatttgcagaagctatatgct

SEQ ID NO: 16 - DNA, 17 bp, Artificial Sequence
  3817 F primer
gagtataagaaggcagt

SEQ ID NO: 17 - DNA, 17 bp, Artificial Sequence
  4553 F primer
tcactatctttaatgag

SEQ ID NO: 18 - DNA, 23 bp, Artificial Sequence
  5455 F primer
ccatttggatgcccagtttatat

SEQ ID NO: 19 - DNA, 17 bp, Artificial Sequence
  R 5583 primer
ctgatgagaatggtgct

SEQ ID NO: 20 - DNA, 25 bp, Artificial Sequence
  Q3’25nts primer
ttgtagcactatgctagtatcagaa

SEQ ID NO: 21 - DNA, 17 bp, Artificial Sequence
  L-segment end q3'R primer
ttgtagcactatgctag

SEQ ID NO: 22 - DNA, 27 bp, Artificial Sequence
  (-2)Rtsm1 primer
gttttattaacaattctaacctcggtt

SEQ ID NO: 23 - DNA, 19 bp, Artificial Sequence
  MRV1ag primer
caaatgactaccagtcagc

SEQ ID NO: 24 - DNA, 24 bp, Artificial Sequence
  RTsm2 primer
caagtgaacagggaaataggatgg

SEQ ID NO: 25 - DNA, 24 bp, Artificial Sequence
  Sm2 primer
gaacatgctgatgcatatgagaca

SEQ ID NO: 26 - DNA, 24 bp, Artificial Sequence
  Sm3 primer
gacccatccttattgtgggcagag

SEQ ID NO: 27 - DNA, 22 bp, Artificial Sequence
  Sm4 primer
atctggcaaaagacgattacgc

SEQ ID NO: 28 - DNA, 18 bp, Artificial Sequence
  EM-RVFV-R primer
cacaaagaccggtgcaac

SEQ ID NO: 29 - DNA, 20 bp, Artificial Sequence
  EM-RVFV-F primer
gaatcaacagttgtgaatcc

SEQ ID NO: 30 - DNA, 19 bp, Artificial Sequence
  NS0g primer
acacaaagaccccctagtg

SEQ ID NO: 31 - DNA, 20 bp, Artificial Sequence
  NS2g primer
tgatttgcagagtggtcgtc

SEQ ID NO: 32 - DNA, 22 bp, Artificial Sequence
  R-S primer
cggacttggagactttgcatca

SEQ ID NO: 33 - DNA, 24 bp, Artificial Sequence
  F-S primer
ttctttcagattggggaaccttgt

SEQ ID NO: 34 - DNA, 18 bp, Artificial Sequence
  NScag primer
ccttaacctctaatcaac

SEQ ID NO: 35 - DNA, 23 bp, Artificial Sequence
  SS1 primer
agccacttaggctgctgtcttgt

SEQ ID NO: 36 - DNA, 30 bp, Artificial Sequence
  RTss1 primer
ctattacaataatggacaactatcaagagc

SEQ ID NO: 37 - DNA, 21 bp, Artificial Sequence
  NP0ag primer
acacaaagctccctagagata

SEQ ID NO: 38 - DNA, 18 bp, Artificial Sequence
  LsegcARN primer
agttttgataatcatgtc

SEQ ID NO: 39 - DNA, 16 bp, Artificial Sequence
  LsegvARN primer
cttttgatacatctga

SEQ ID NO: 40 - DNA, 17 bp, Artificial Sequence
  MsegcARN primer
gtttctctccctatttg

SEQ ID NO: 41 - DNA, 18 bp, Artificial Sequence
  MsegvARN primer
tcctccttatatatcttg

SEQ ID NO: 42 - DNA, 18 bp, Artificial Sequence
  SsegcARN primer
tattagatcaataagtct

SEQ ID NO: 43 - DNA, 17 bp, Artificial Sequence
  SsegvARN primer
tctttcgacattttcat

SEQ ID NO: 44 - DNA, 6404 bp, Artificial Sequence
  RVFV 56/74 L segment
  gene 19..6297: /note="RVFV 56/74 L segment open reading frame"
acacaaaggcgcccaatcatggattctatattatcaaaacagctggttgacaagactggttttgttagagtgccaatcaagcattatgactgtacaatgctaactctggcactcccaacatttgatgtctccaagatggtagatagaattaccatagacttcaatttagacgacatacaaggagcatctgaaataggctcaactttgctaccctctatgtcgatagatgtggaagatatggccaattttgttcacgatttcacctttggccacttagctgacaagactgacagactcttaatgcgtgagtttcccatgatgaatgacgggtttgatcatctgagccctgacatgattatcaaaactacatctggcatgtataacatcgttgagttcaccacctttaggggggatgaaagaggtgcattccaggctgccatgactaaactcgctaagtatgaggttccttgtgagaacagatctcagggcaggactgttgttctttatgttgttagcgcctaccggcatggtgtttggtctaatttggagctagaggactctgaagcagaggagatggtatataggtacagacttgcccttagtgtgatggatgagctaaggaccttgttcccagaactgtcatccacagatgaggaactaggaaagactgagagagagttgctagccatggtctcctccatccaaataaattggtcagtcacagaatctgtgtttcctccctttagcagagaaatgtttgacaggttcagatcttctcctcccgattcagagtacatcacgaggatagtgagcagatgcctcataaattctcaagagaaactcatcaataattccttctttgctgaagggaatgataaagttttgagattttcaaaaaacgctgaggagtgttccttggcaatagagagagctttaaatcagtatagggcagaagacaaccttagggacctcaatgaccacaagtctactattcagctgcccccctggctgtcctatcacgatgccgatggcaaagatctgtgccctcttcagggattagatgtgagaggagaccatcccatgtgcaacctgtggagagaagtggttacctctgcaaatctagaggagattgagaggatgcacgatgatgcagcggcagaacttgagtttgccctttcaggggtgaaggacaggccagatgaaagaaacagataccatagagtccatctgaatatggactcagatgatagtgtctacatagctgctttaggggttaatggaaagaagcataaagcagacacattagtgcaacaaatgagagacaggagcaaacagcccttctctccagatcatgatgtggatcacatatctgaatttctctctgcatgctctagtgacttgtgggcaacagatgaggacctatacaaccctctctcttgtgataaagagcttagattggcagctcagagaattcatcagccatccttatcagaaaggggcttcaatgagattataacagagcactacagatttatgggaagtaggataggatcatggtgccaaatggtcagtttaataggagctgagctatcagcttctgtaaagcaacatgttaagcctaactattttgtgattaaacgactactaggttctgggattttcttgctgatcaagcctacttccagcaaaagccatatattcgtgtcttttgcaattaagcgctcttgctgggcctttgatctctccacttccagggttttcaaaccctacatagatgccggggatctgttagttactgactttgtttcttacaaactaagtaagcttaccaacctctgcaagtgcgtttcgttaatggaatcctccttctcattttgggcagaggcatttgggattccaagctggaactttgttagtgacttgttcaggtcttcagactctgcagcaatggatgcctcatacatgggcaaactctctttattaacccttttggaagacaaagcaacaactgaagagttacagactattgcaagatatataatcatggagggctttgtctcgcccccagaaatcccaaaacctcacaagatgacctctaagtttcccaaggttctcaggtcagagctgcaggtttacttattaaactgcttatgcagaactatccagagaatagcaggtgagccctttattcttaagaagaaggatgggtctatatcctggggtggcatgtttaatcctttttcagggcgtccactgcttgatatgcaaccactcatcagctgttgttacaatggttactttaaaaacaaagaagaagagactgagccttcctccctttctgggatgtataagaaaattatagaacttgagcaccttagaccacagtcagatgccttcttgggttataaagatccagaactacctagaatgcatgagttcagtgtttcctacttgaaggaggcttgcaatcatgctaagctggtcttaaggagtctctatggacagaatttcatggagcaaatagacaaccaaattattcgagagctcagtgggttgactctagaaagattagccacacttaaggccacaagcaactttaatgagaattggtatgtctataaggatgtggcagacaagaactacacaagggataaattattagtgaagatgtcaaaatatgcttctgagggaaagagcctagctatccagaagtttgaggattgcatgaggcagatagagtcacaaggatgtatgcacatttgtttgtttaagaaacaacagcatggaggtctgagagagatctatgtgatgggtgcagaggaaagaattgttcaatcggtggtggagacaatagccaggtctatagggaagttctttgcttctgataccctctgtaacccccccaataaggtgaaaattcctgagacacatggcattagggctcggaagcaatgtaaggggcctgtgtggacttgtgcaacatcagatgatgcaaggaagtggaaccaaggccattttgttacaaagtttgccctcatgctatgtgagttcacctctcctaagtggtggccattgatcattaggggatgttcaatgtttaccaggaaaaggatgatgatgaatttgaattatcttaagatcctggatggtcatcgagagcttgatattagagatgactttgtgatggatctcttcaaagcttatcatggtgaggcagaagttccatgggcttttaagggtaaaacatatctggaaaccacaacagggatgatgcaggggatattgcattatacttcctcattattacacaccattcatcaagaatacatccggtccttgtcctttaaaatattcaacctgaaggttgctcctgagatgagcaaaagcctggtttgtgacatgatgcaaggatcagatgatagtagcatgctaatcagcttcccagctgatgacgagaaggttctcaccagatgcaaagtggccgcagccatatgcttccgaatgaagaaggagctgggagtgtaccttgccatctacccctcagagaagtccacagcaaacacagattttgtgatggagtacaattctgaattttatttccacacccagcatgttagaccgacgatcaggtggattgcagcatgttgcagcctgccagaagtggaaacactagtagcccgccaggaagaggcctctaatctaatgacttcagttactgaggggggtgggtcattctccttagctgcaatgattcagcaagctcagtgcactctccattacatgctaatgggcatgggagtgtctgagctattcttagagtataagaaggcagtgctgaagtggaatgaccctggtctgggtttcttcctgcttgacaatccttatgcgtgcgggttgggaggttttagatttaatctcttcaaagccatcaccagaactgatttgcagaagctatatgctttcttcatgaagaaggttaagggctcagctgctagggactgggcagatgaggatgttaccatcccagaaacgtgtagcgtgagcccaggtggcgctctaattcttagctcctctctaaagtggggatctaggaagaagtttcagaaactgagagaccgtttgaacataccagagaactggattgagctaataaatgagaatccagaggtgctctatcgagctcccagaacaggcccagaaatattgttgcgcattgcagagaaagtccatagccctggtgttgtgtcatcattgtcttctggcaatgcagtctgtaaagtcatggcctcagctgtatacttcttatcagcaacaatttttgaagacactggacgccctgagttcaacttcttagaggattccaagtacagcttgctacaaaagatggccgcatattctggctttcatggtttcaatgatatggagccagaagatatattattcctattcccgaacattgaggaattagaatcactggattctatagtttacaacaagggagaaatagacatcatcccaagagttaatatcagggatgcaacccaaaccagggtcactatctttaatgagcagaagaccctccgaacatctccagagaagttggtgtcagacaagtggttcgggactcagaagagtaggataggcaaaacaactttcctggctgaatgggagaagctaaagaaaattgtgaagtggttggaagacactccagaagcaactctagctcacactccactgaataaccatattcaggttaggaatttctttgctagaatggaaagcaagcctagaacggttagaataacaggagctcctgtaaagaagaggtcaggggttagcaagatagctatggttatccgtgacaatttctcccggatgggccatcttagaggtgtagaagacctcgctggcttcactcgtagtgtgtcagctgaaatcctcaagcactttctgttctgcatactacagggtccatacagtgagagctataagctacagctaatctacagagtcctaagctcagtgtcaaacgttgagataaaggaatcggatggtaagacaaaaaccaatttgattgggatccttcagagatttctagatggtgatcacgttgtccctataattgaagagatgggagccggaacagtgggtggattcatcaagagacaacagtctaaggttgtgcaaaataaagtggtctattatggagttgggatctggagaggcttcatggatggatatcaggtccatcttgagatagaaaatgacataggacagcccccaaggcttaggaatgtcacaactaactgtcagagcagcccatgggatctgagtgtcccaataaggcagtgggcagaagacatgggggtcacaaacaaccaggattattcctctaaatctagcagaggagctagatattggatgcattcatttaggatgcaaggacccagcaagccatttggatgcccagtttatattattaagggtgacatgtcagatgttatcagactgagaaaagaggaggtggagatgaaagtacggggctctactctcaacttgtacactaagcaccattctcatcaagacttacacattttatcttacactgcatcagacaatgatctcagtccaggcattttcaagtcaatatcagatgagggagtggctcaagccctgcagttatttgagagggagccaagcaactgctgggtgagatgtgagtctgtagctccaaaattcatatcagccatccttgagatatgtgaggggaagagacagataaaaggaatcaacagaaccagactctcagagattgtgagaatttgttctgaatcttccctaagatcaaaggtcggatctatgttctcatttgtcgccaatgttgaggaggcccatgatgttgattatgatgcgttaatggatctaatgatagaagatgctaagaacaatgcattcagtcatgttgtcgattgcatagagttggatgttaatggtccttacgagatggagtcttttgatacatctgatgtcaacctctttgggccagcccattacaaggacatcagttcattatctatgattgctcatcccttaatggataagtttgttgattatgccatttccaagatggggagagcctcagttagaaaagttctagagacaggtcggtgctctagcaaagactatgatttatcaaaggttctcttcagaactctacagagaccagaagagagcattaggatagatgatctggagttatatgaggagacagatgtggcggatgacatgctaggctaagaccaataagcaaagtcaggcttagatttagggatactacgctagtattggaatccatgtgggttctgatactagcatagtgctacaatattgggcggtctttgtgt

SEQ ID NO: 45 - DNA, 3885 bp, Artificial Sequence
  RVFV 56/74 M segment
  gene 21..3614: /note="RVFV 56/74 gene encoding M (poly)protein"
acacaaagacggtgcattaaatgtatgttttactaacaattctgatcacggttctggtgtgtgaagcggttattagagtgtctctaagctccacaagagaagagacctgttttggtgactccaccaacccagagatgattgaaggagcttgggattcactcagagaggaggagatgccagaggagctctcctgttctatatcaggcataagggaggttaagacctcaagccaggagttatacagggcattaaaagccatcattgctgctgatggcttgaacaacatcacctgccatggtaaggatcctgaggacaagatttctctcataaagggtcctcctcacaaaaagcgggtggggatagttcggtgtgagagacgaagagatgctaagcaaatagggagagaaaccatggcagggattgcaatgacagtccttccagccttagcagtttttgctttggcacctgttgtttttgctgaagacccccatctcaggaacagaccagggaaggggcacaactacattgacgggatgactcaggaggatgccacatgcaaacctgtgacatatgctggggcatgtagcagttttgatgtcttgcttgaaaaggggaaatttccccttttccagtcgtatgctcatcatagaactctactggaagcagttcacgacactatcattgcaaaggctgatccacctagctgtgaccttcagagtgctcatgggaatccctgcatgaaagagaaactcgtgatgaagacacactgtccaaatgactaccagtcagctcattacctcaacaatgacgggaaagtggcttcagtcaagtgccctcctaagtatgagctcactgaggactgcaacttttgtaggcagatgacaggtgctagcctgaagaaagggtcttatcctctccaagacttattttgtcagtcaagtgaggatgatggatcaaaattaaaaacaaaaatgaaaggggtctgcgaagtgggggttcaagcactcaaaaagtgtgatggccaactcagcactgcacatgaggttgtgccctttgcagtgtttaagaactcaaagaaagtttatcttgataagcttgacctcaaaactgaggagaatctgctaccagactcatttgtctgcttcgagcataagggacagtataaaggaacaatggactctggtcagactaagagggagctcaaaagctctgatatctctcagtgccccaagattggaggacatggtagtaaaaagtgcactggggacgcagcattttgctctgcttatgagtgcactgctcagtacgccaatgcctactgttcacatgctaatggttcagggattgtgcagatacaagtatcaggggtctggaagaagcctttatgtgtagggtatgagagagtggttgtgaagagagaactctctgccaagcccatccagagagttgagccctgcacaacttgtataaccaaatgtgagcctcatggattggttgtccgatcaacagggttcaagatatcatctgcagttgcttgtgctagcggagtttgcgtcacaggatcgcagagtccttctaccgagattacactcaagtatccagggatatcccagtcctctgggggggacataggggttcacatggcacatgatgatcagtcagttagctccaaaatagtagctcactgccccccccaggacccgtgcttagtgcatggctgcatagtgtgtgctcatggcctgataaattaccagtgtcacactgctctcagtgcctttgttgttgtgtttgtattcagttctattgcaataacttgtttagctattctttatagggtgctcaagtgcctaaagattgccccaaggaaggttctaaatccactaatgtggattacagccttcatcagatgggtgtataagaagatggttgctagagtggcagacaatattaatcaagtgaacagggaaataggatggatggaagggggtcagttggttctagggaaccctgcccctattcctcgtcatgccccaatcccacgttatagcacatacctaatgctactattgattgtctcatatgcatcagcatgttcagaactgattcaggcaagctccagaatcaccacttgctccacagagggtgttaacaccaagtgtagactgtctggcacagcattgatcagggcagggtcagttggggcagaggcttgtttaatgttgaagggggtcaaggaagatcaaaccaaattcttgaagataaaaactgtctcaagtgagctatcgtgcagggagggccagagctattggactgggtcctttagccccaaatgtctgagctcaaggagatgccatcttgttggagaatgtcatgtgaataggtgtctgtcttggagggacaatgaaacttcagcagagttttcatttgttggggaaagcacgaccatgcgagagaataagtgttttgagcagtgtggaggatgggggtgtgggtgcttcaatgtgaacccatcttgcttatttgtgcacacgtacctgcagtcagttagaaaagaggcccttagagtttttaactgtatcgactgggtgcataaactcagtctagagatcacagactttgatggctctgtttcaacaatagacttgggagcatcatctagccgtttcacaaactggggttcagttagcctctcactggacgcagagggtatttcaggctcaaatagcttttctttcattgagagcccaggcaaagggtatgcaattgttgatgagccattctcagaaattcctcggcaagggttcttgggggagatcaggtgtaattcagagtcctcagtcctgagtgctcatgaatcatgccttagggcaccaaaccttatctcatacaagcccatgatagatcaattggagtgcacaacaaatctgattgatccttttgttgtctttgagaggggttctctgccacagacaaggaatgaaaaaacctttgcagcttcaaaaggaaataggggtgttcaagctttctctaagggctctgtacaagctgatctaactctgatgtttgacaattttgaggtggactttgtgggagcagccgtatcttgtgatgccgccttcttaaacttgacaggttgctattcttgcaatgcgggagccagggtctgcctgtctatcacatccacaggaactggaactctctctgcccacaataaggatgggtctctgcacatagttcttccatcagagaatggaacaaaagatcagtgtcagatactacacttcactgtacctgaagtagaggaggagtttatgtactcttgtgatggagatgagcggcctctgttggtgaaagggaccctgatagctattgatccatttgatgataggcgggaagcagggggggaatcaacagttgtgaatccaaaatctggatcttggaatttctttgactggttttctggactcatgagttggtttggagggcctcttaaaactatactcctcatttgcctgtatgttgcattatcaattgggctctttttcctccttatatatcttggaagaacaggcctctctaaaatgtggcttgctgctactaagaaggcctcatagatcagtacgtgtagaagcaatatgtagaaacaagtggacataagcaaacctaattatgtaaatattgtacagataggtcaaattattgggatatccaagcttagatgcttatgcaatattacttttgatgtaagcttagttgtaatttggggtggtggggtgaggcagcagcagtctcaagtgcttgtgaatattctagttggcgtaattgtcttttgccagattagctgggaattaaactaactctttgaagttgcaccggtctttgtgt

SEQ ID NO: 46 - DNA, 1691 bp, Artificial Sequence
  RVFV 56/74 S segment
  gene 35..832: /note="RVFV 56/74 gene encoding NSs protein"
  gene 916..1653: /note="RVF virus gene encoding N protein 56/74"
acacaaagaccccctagtgcttatcaagtgtatcatggattactttcctgtgatatctgttgatttgcagagtggtcgtcgtgttgtgtcagtggagtacattagaggtgatggtcctcccaggataccttattctatggttgggccctgttgtgtctttctcatgcaccatcgtcctagtcacgaggttcgcttgcgattctctgatttctacaatgtcggagaattcccataccgagtcggacttggagactttgtatcaaacgttgcacctccaccagcaaagccttttcagagacttattgatctaataggccatatgactcttagtgatttcacaaggttccccaatctgaaagaagccatatcctggcctcttggagaaccctccctggctttctttgacctaagctccaccagagtgcataggtctgatgatattagaagggaccagattgctactctagcaatgaggagctgcaagattaccaatgatctggaggactcctttgttggcttacacaggatgatagtgaccgaggctatcctcagagggattgacttgtgcctgttgccaggctttgatctcatgtatgaggttgctcacgttcagtgtgttcggctcctgcaggcagcaagagaggatatttctaatgctgtagttccaaactcagctctcattgctcttatggaggagagcttgatgctgcgctcatcactccctagcatgatggggagaaacaactgggttccagttgttcctccaatcccagatgttgagatagaatcagaggaagagagtgatgacgatggatttgttgaggttgattagagattaaggctgccccaccccccacccccaatcccgaccgtaaccccaaccacccccttttccccaaacccctgggcagccacttaggctgctgtcttgtacgcctgagcagctgccatgacagctgctgacggcttcccattggaatccacaagcccaaaagctttcaagaattctctcctcttctcatggcttataaagttgctattcactgctgcattcattggctgcgtgaacgttgcggcaacctcctcctttgttctacctcggaggtttgggttgatgacccgggagaactgcagcagatacagagagtgagcatccaatattgcccttagatagtcttctggtagagaagggtccaccatgccagcaaagctggggtgcatcatatgccttgggtatgcaggggataggccatccatggtggtcccagtgacaggaagccactcactcaagacgaccaaagcctggcaagtccagccagccagggcagcagcaactcgtgatagagtcaactcatcccgggaaggattcccctcctttagcttatacttgttgatgagagcctccacagttgctttgccttctttcgacattttcatcatcatcctccggggcttgttgccacgagtcagagccagaacaatcattttcttggcatccttctcccagccagccccaccatactgctttaagagttcgataaccctacgggcatcaaatccttgataagcaaactctcggacccactgttcaatctcattgcggtccactgcttgagcagcaaactggatcgcaagctcttgatagttgtccattattgtaatagtgtttgtatctctagggagctttgtgt

SEQ ID NO: 47 - protein, 2092 aa, Artificial Sequence
  RVFV 56/74 L protein
MDSILSKQLVDKTGFVRVPIKHYDCTMLTLALPTFDVSKMVDRITIDFNLDDIQGASEIGSTLLPSMSIDVEDMANFVHDFTFGHLADKTDRLLMREFPMMNDGFDHLSPDMIIKTTSGMYNIVEFTTFRGDERGAFQAAMTKLAKYEVPCENRSQGRTVVLYVVSAYRHGVWSNLELEDSEAEEMVYRYRLALSVMDELRTLFPELSSTDEELGKTERELLAMVSSIQINWSVTESVFPPFSREMFDRFRSSPPDSEYITRIVSRCLINSQEKLINNSFFAEGNDKVLRFSKNAEECSLAIERALNQYRAEDNLRDLNDHKSTIQLPPWLSYHDADGKDLCPLQGLDVRGDHPMCNLWREVVTSANLEEIERMHDDAAAELEFALSGVKDRPDERNRYHRVHLNMDSDDSVYIAALGVNGKKHKADTLVQQMRDRSKQPFSPDHDVDHISEFLSACSSDLWATDEDLYNPLSCDKELRLAAQRIHQPSLSERGFNEIITEHYRFMGSRIGSWCQMVSLIGAELSASVKQHVKPNYFVIKRLLGSGIFLLIKPTSSKSHIFVSFAIKRSCWAFDLSTSRVFKPYIDAGDLLVTDFVSYKLSKLTNLCKCVSLMESSFSFWAEAFGIPSWNFVSDLFRSSDSAAMDASYMGKLSLLTLLEDKATTEELQTIARYIIMEGFVSPPEIPKPHKMTSKFPKVLRSELQVYLLNCLCRTIQRIAGEPFILKKKDGSISWGGMFNPFSGRPLLDMQPLISCCYNGYFKNKEEETEPSSLSGMYKKIIELEHLRPQSDAFLGYKDPELPRMHEFSVSYLKEACNHAKLVLRSLYGQNFMEQIDNQIIRELSGLTLERLATLKATSNFNENWYVYKDVADKNYTRDKLLVKMSKYASEGKSLAIQKFEDCMRQIESQGCMHICLFKKQQHGGLREIYVMGAEERIVQSVVETIARSIGKFFASDTLCNPPNKVKIPETHGIRARKQCKGPVWTCATSDDARKWNQGHFVTKFALMLCEFTSPKWWPLIIRGCSMFTRKRMMMNLNYLKILDGHRELDIRDDFVMDLFKAYHGEAEVPWAFKGKTYLETTTGMMQGILHYTSSLLHTIHQEYIRSLSFKIFNLKVAPEMSKSLVCDMMQGSDDSSMLISFPADDEKVLTRCKVAAAICFRMKKELGVYLAIYPSEKSTANTDFVMEYNSEFYFHTQHVRPTIRWIAACCSLPEVETLVARQEEASNLMTSVTEGGGSFSLAAMIQQAQCTLHYMLMGMGVSELFLEYKKAVLKWNDPGLGFFLLDNPYACGLGGFRFNLFKAITRTDLQKLYAFFMKKVKGSAARDWADEDVTIPETCSVSPGGALILSSSLKWGSRKKFQKLRDRLNIPENWIELINENPEVLYRAPRTGPEILLRIAEKVHSPGVVSSLSSGNAVCKVMASAVYFLSATIFEDTGRPEFNFLEDSKYSLLQKMAAYSGFHGFNDMEPEDILFLFPNIEELESLDSIVYNKGEIDIIPRVNIRDATQTRVTIFNEQKTLRTSPEKLVSDKWFGTQKSRIGKTTFLAEWEKLKKIVKWLEDTPEATLAHTPLNNHIQVRNFFARMESKPRTVRITGAPVKKRSGVSKIAMVIRDNFSRMGHLRGVEDLAGFTRSVSAEILKHFLFCILQGPYSESYKLQLIYRVLSSVSNVEIKESDGKTKTNLIGILQRFLDGDHVVPIIEEMGAGTVGGFIKRQQSKVVQNKVVYYGVGIWRGFMDGYQVHLEIENDIGQPPRLRNVTTNCQSSPWDLSVPIRQWAEDMGVTNNQDYSSKSSRGARYWMHSFRMQGPSKPFGCPVYIIKGDMSDVIRLRKEEVEMKVRGSTLNLYTKHHSHQDLHILSYTASDNDLSPGIFKSISDEGVAQALQLFEREPSNCWVRCESVAPKFISAILEICEGKRQIKGINRTRLSEIVRICSESSLRSKVGSMFSFVANVEEAHDVDYDALMDLMIEDAKNNAFSHVVDCIELDVNGPYEMESFDTSDVNLFGPAHYKDISSLSMIAHPLMDKFVDYAISKMGRASVRKVLETGRCSSKDYDLSKVLFRTLQRPEESIRIDDLELYEETDVADDMLG

SEQ ID NO: 48 - protein, 1197 aa, Artificial Sequence
  RVFV 56/74 M poly(protein)
MYVLLTILITVLVCEAVIRVSLSSTREETCFGDSTNPEMIEGAWDSLREEEMPEELSCSISGIREVKTSSQELYRALKAIIAADGLNNITCHGKDPEDKISLIKGPPHKKRVGIVRCERRRDAKQIGRETMAGIAMTVLPALAVFALAPVVFAEDPHLRNRPGKGHNYIDGMTQEDATCKPVTYAGACSSFDVLLEKGKFPLFQSYAHHRTLLEAVHDTIIAKADPPSCDLQSAHGNPCMKEKLVMKTHCPNDYQSAHYLNNDGKVASVKCPPKYELTEDCNFCRQMTGASLKKGSYPLQDLFCQSSEDDGSKLKTKMKGVCEVGVQALKKCDGQLSTAHEVVPFAVFKNSKKVYLDKLDLKTEENLLPDSFVCFEHKGQYKGTMDSGQTKRELKSSDISQCPKIGGHGSKKCTGDAAFCSAYECTAQYANAYCSHANGSGIVQIQVSGVWKKPLCVGYERVVVKRELSAKPIQRVEPCTTCITKCEPHGLVVRSTGFKISSAVACASGVCVTGSQSPSTEITLKYPGISQSSGGDIGVHMAHDDQSVSSKIVAHCPPQDPCLVHGCIVCAHGLINYQCHTALSAFVVVFVFSSIAITCLAILYRVLKCLKIAPRKVLNPLMWITAFIRWVYKKMVARVADNINQVNREIGWMEGGQLVLGNPAPIPRHAPIPRYSTYLMLLLIVSYASACSELIQASSRITTCSTEGVNTKCRLSGTALIRAGSVGAEACLMLKGVKEDQTKFLKIKTVSSELSCREGQSYWTGSFSPKCLSSRRCHLVGECHVNRCLSWRDNETSAEFSFVGESTTMRENKCFEQCGGWGCGCFNVNPSCLFVHTYLQSVRKEALRVFNCIDWVHKLSLEITDFDGSVSTIDLGASSSRFTNWGSVSLSLDAEGISGSNSFSFIESPGKGYAIVDEPFSEIPRQGFLGEIRCNSESSVLSAHESCLRAPNLISYKPMIDQLECTTNLIDPFVVFERGSLPQTRNEKTFAASKGNRGVQAFSKGSVQADLTLMFDNFEVDFVGAAVSCDAAFLNLTGCYSCNAGARVCLSITSTGTGTLSAHNKDGSLHIVLPSENGTKDQCQILHFTVPEVEEEFMYSCDGDERPLLVKGTLIAIDPFDDRREAGGESTVVNPKSGSWNFFDWFSGLMSWFGGPLKTILLICLYVALSIGLFFLLIYLGRTGLSKMWLAATKKAS

SEQ ID NO: 49 - protein, 265 aa, Artificial Sequence
  RVFV 56/74 NSs protein
MDYFPVISVDLQSGRRVVSVEYIRGDGPPRIPYSMVGPCCVFLMHHRPSHEVRLRFSDFYNVGEFPYRVGLGDFVSNVAPPPAKPFQRLIDLIGHMTLSDFTRFPNLKEAISWPLGEPSLAFFDLSSTRVHRSDDIRRDQIATLAMRSCKITNDLEDSFVGLHRMIVTEAILRGIDLCLLPGFDLMYEVAHVQCVRLLQAAREDISNAVVPNSALIALMEESLMLRSSLPSMMGRNNWVPVVPPIPDVEIESEEESDDDGFVEVD

SEQ ID NO: 50 - protein, 245 aa, Artificial Sequence; identical to SEQ ID NO: 7
  RVFV 56/74 N protein

SEQ ID NO: 51 - DNA, 6404 bp, Artificial Sequence
  ZH548 RVF virus L segment
  gene 19..6297: /note="ZH548 RVF virus L-segment open reading frame"
acacaaaggcgcccaatcatggattctatattatcaaaacagctggttgacaagactggttttgttagagtgccaatcaagcattttgactgtacaatgctaactctggcacttccaacatttgatgtttccaagatggtagatagaattaccatagacttcaatctggatgatatacaaggagcatctgaaataggctcaactttgctaccctccatgtcgatagatgtggaagatatggccaattttgttcacgatttcacctttggccacttagctgacaagactgacagactgttaatgcgtgagtttcccatgatgaatgacgggtttgatcatttgagccctgacatgatcattaaaactacatctggcatgtacaacatcgttgagttcaccacctttaggggagatgaaagaggtgcattccaggctgccatgactaaactcgctaagtatgaggttccttgtgagaacagatctcagggcaggactgttgttctttatgttgttagtgcttatcggcatggtgtatggtctaatctggagctagaggactctgaagcagaggagatggtttataggtacagacttgctcttagtgtgatggatgagctaaggaccttgttcccagaactgtcatccacagatgaggaactagggaagactgagagagagttgctagccatggtctcctccatccaaataaattggtcagtcacagaatctgtgtttccacccttcagcagagaaatgtttgacaggtttagatcctcccctcccgattcagagtatatcacgaggatagtgagcagatgcctaataaattctcaagagaaactcatcaatagttccttctttgctgaagggaatgataaggctctgagattttcaaaaaacgctgaagagtgttccttggcagtagagagagccttaaatcagtatagagcagaagacaaccttagggacctcaatgaccacaagtcaactattcagctgcctccctggctgtcctatcatgatgtcgatggcaaagatctgtgccctcttcagggactagatgtgagaggggaccatcccatgtgcaacttgtggagggaagtggtcacctctgcaaacctagaggagattgagaggatgcacgatgatgcagcagcagaacttgagtttgccctttcgggagtaaaggacaggccagatgagagaaacagataccatagagtccacctaaatatgggctcagatgatagtgtctacatagctgctttaggagttaatggaaagaagcataaagcagacactttagtgcaacaaatgagagacaggagtaaacagcctttctccccagaccacgatgtggatcacatatctgaatttctctctgcatgctctagtgacttgtgggcaacagatgaggacctgtacagccctctctcttgtgataaagagcttagattggcagcccagaggattcatcagccatccttgtcagaaaggggtttcaatgagatcataacagagcactacaaattcatgggaagtaggataggttcatggtgccaaatggtcagcttgataggagctgagctatcagcttctgttaaacaacatgtcaagcctaactactttgtgattaaacgactactaggttctgggattttcttgctaatcaagcccacttccagcaaaagccatatatttgtgtcttttgcaattaagcgctcttgctgggcctttgatctctccacttccagggttttcaagccctacatagatgctggggatctgttagttactgactttgtttcttataagctaagcaagcttaccaacctctgcaagtgcgtttcattaatggagtcctccttctcattctgggcagaagcatttggaattccaagctggaactttgttggtgacttgttcaggtcttcagactctgcagcaatggatgcctcatacatgggcaaactttctttattaacccttttggaagacaaagcagcaactgaagagttacagactattgcaagatatataatcatggagggctttgtctcgcccccagaaatcccaaaacctcacaagatgacctctaagtttcctaaggttctcaggtcagagctgcaggtttacttattaaactgcttatgcagaactatccagagaatagcaggtgagcccttcattcttaagaagaaggatgggtctatatcctggggtggcatgttcaatcctttttcagggcgtccactgcttgatatgcaaccactcatcagctgttgttacaatggttactttaaaaataaagaagaagagactgagccttcgtccctttctgggatgtataagaaaatcatagaacttgagcaccttagaccacagtcagatgccttcttgggttacaaagatccagaacttcccagaatgcatgagttcagtgtttcctacttgaaggaggcttgcaatcatgctaagctagtcttgaggagcctctatggacagaatttcatggagcagatagacaaccagattattcgagagctcagtgggttgactctagaaaggttggccacacttaaggccacaagcaactttaatgagaattggtatgtctataaggatgtagcagacaaaaactacacaagggataaattattagtgaagatgtcaaaatatgcctctgagggaaagagcctagctatccagaagtttgaggattgtatgaggcagatagagtcacaaggatgcatgcatatttgtttgtttaagaaacaacagcatggaggtctgagagagatctatgtgatgggtgcagaggaaagaattgttcaatcggtggtggagacaatagccaggtccatagggaagttctttgcttctgataccctctgtaacccccccaataaagtgaaaattcctgagacacatggcatcagggcccggaagcaatgtaaggggcctgtgtggacttgtgcaacatcagatgatgcaaggaagtggaaccaaggccattttgttacaaagtttgccctcatgctgtgtgagttcacctctcctaaatggtggccgctgatcattaggggatgctcaatgtttaccaggaaaaggatgatgatgaatttgaattatcttaagatcctggatggtcatcgggagcttgatattagagatgactttgtgatggatctcttcaaagcttatcatggcgaggcagaagttccatgggcctttaaaggcaaaacatatttggaaaccacaacagggatgatgcagggaatactgcattatacttcctcactattacacaccattcaccaagaatacatccggtccttgtcctttaagatattcaacctgaaggttgctcctgagatgagcaagagcctggtttgtgacatgatgcaaggatcagatgatagtagtatgctaatcagcttcccagctgatgatgagaaggttcttaccagatgcaaagtggccgcagctatatgcttccgcatgaagaaggagctgggagtgtaccttgccatttacccctcagagaagtccacagcaaacacagattttgtgatggagtacaattctgaattttatttccacacccagcatgttagaccaacgatcaggtggattgcagcttgttgcagcctgccagaagtggaaacactagtagcccgccaggaagaggcctctaacctaatgacttcagttactgagggaggtgggtcattctccttagctgcaatgattcagcaagctcagtgtactctccattacatgctgatgggcatgggagtgtctgagctattcttagagtataagaaggcagtgctgaagtggaatgaccctggcctgggtttcttcctgcttgacaatccttatgcgtgcggattgggaggtttcagatttaatctcttcaaagctatcaccagaactgatttgcagaagctatatgctttcttcatgaagaaggtcaagggctcagctgctagggactgggcagatgaagatgtcaccatcccagaaacgtgtagcgtgagcccaggtggcgctctaattcttagctcctctctaaagtggggatctaggaagaagtttcagaaattgagagaccgtttgaacataccagagaactggattgaactaataaatgagaatccagaggtgctctatcgggctcccagaacaggcccagaaatattgttgcgcattgcagagaaagtccatagcccaggtgttgtgtcatcattgtcttctggcaatgcagtttgtaaagtcatggcctcagctgtatacttcttatcagcaacaatttttgaggacactggacgtcctgagttcaacttcttggaggattctaagtacagcttgctacaaaagatggctgcatattctggctttcatggtttcaatgatatggagccagaagatatattattcttattcccgaatattgaggaattagaatcactggattctatagtttacaacaagggagaaatagacatcatcccaagagtcaacatcagggatgcaacccaaaccagggtcactatctttaatgagcagaagaccctccggacatctccagagaagttggtgtcagacaagtggtttgggactcagaagagtaggataggcaaaacaaccttcctggctgaatgggaaaagctaaagaaaattgtaaagtggttggaagacactccagaagcaactctagctcacaccccactgaataaccatattcaagttaggaatttctttgctagaatggaaagcaagcctagaacagtcagaataacaggagctccagtaaagaagaggtcaggggttagtaagatagctatggttatccgtgacaatttctcccggatgggccatcttcgaggtgtagaagaccttgctggcttcactcgtagtgtgtcagctgaaattctcaagcactttctattctgtatactacaaggtccatacagtgagagctataagctacagctaatctacagagtcctaagctcagtgtcaaacgttgagataaaggaatcagatggtaagacaaaaaccaacttgattggaatccttcagagatttctagatggtgatcacgttgtccccataattgaagagatgggagccggaacagtgggtggattcatcaagagacaacaatctaaagttgtgcagaacaaagtggtctattatggagttgggatttggagaggcttcatggatggatatcaggtccatctagagatagaaaatgacataggacagcccccaaggcttaggaatgtcacaactaactgtcagagcagcccatgggacctgagtattccaataaggcaatgggcagaagacatgggggtcacaaacaaccaggattattcctctaaatctagcaggggggccagatattggatgcattcattcaggatgcaaggacctagcaagccatttggatgcccagtttatattattaagggtgatatgtcagatgtcatcagactgagaaaggaggaggtggagatgaaagtacggggctctactctcaacttgtacaccaagcaccattctcatcaggacctacacattctatcttacactgcatcagacaatgatctcagtccaggcattttcaagtcaatatcagatgagggggtggctcaagccctgcaattatttgagagggagccaagcaactgctgggtgagatgtgagtctgtagccccaaaatttatatcagccatccttgagatatgtgaggggaagagacagataaagggaattaacagaaccagactctcagagattgtgagaatttgttctgaatcttccctaagatcaaaagtcggatctatgttctcatttgtcgccaatgtcgaggaggcccatgatgttgattatgatgcgttaatggatctaatgatagaggatgccaagaacaatgcattcagtcatgttgttgactgcatagagttggatgttagtggcccttacgagatggagtcttttgatacatctgatgtcaatctctttgggccagcccattacaaggacatcagttcattatctatgattgctcatcccttaatggataagtttgttgattatgctatttctaagatggggagagcctcagttaggaaagttctagaaacaggtcggtgctccagcaaagactatgatttatcaaaggttctcttcagaactctacagagaccagaagaaagcattaggatagatgatctggaattatatgaggagacagatgtggcggatgacatgctaggctaagaccagtaagcaaagtcaggcttagatttagggatactatgctagtattggaatccatgtgggttctgatactagcatagtgctacaatattgggcggtctttgtgt

SEQ ID NO: 52 - DNA, 3885 bp, Artificial Sequence
  ZH548 RVF virus M segment
  gene 21..3614: /note="ZH548 RFV virus gene encoding M (poly)protein"
acacaaagacggtgcattaaatgtatgttttattaacaattctaatctcggttctggtgtgtgaagcggttattagagtgtctctaagctccacaagagaagagacctgctttggtgactccactaacccagagatgattgaaggagcttgggattcactcagagaggaggagatgccggaggagctctcctgttctatatcaggcataagagaggttaagacctcaagccaggagttatacagggcattaaaagccatcattgctgctgatggcttgaacaacatcacctgccatggtaaggatcctgaggacaagatttccctcataaagggtcctcctcacaaaaagcgggtggggatagttcggtgtgagagacgaagagatgctaagcaaatagggagagaaaccatggcagggattgcaatgacagtccttccagccttagcagtttttgctttggcacctgttgtttttgctgaagacccccatctcagaaacagaccagggaaggggcacaactacattgacgggatgactcaggaggatgccacatgcaaacctgtgacatatgctggggcatgtagcagttttgatgtcttgcttgaaaagggaaaatttccccttttccagtcgtatgctcatcatagaactctactagaggcagttcacgacaccatcattgcaaaggctgatccacctagctgtgaccttctgagtgctcatgggaacccctgcatgaaagagaaactcgtgatgaagacacactgtccaaatgactaccagtcagctcattacctcaacaatgacgggaaaatggcttcagtcaagtgccctcctaagtatgagctcactgaggactgcaacttttgtaggcagatgacaggtgctagcctgaagaaggggtcttatcctctccaagacttgttttgtcagtcaagtgaggatgatggatcaaaattaaaaacaaaaatgaaaggggtctgcgaagtgggggttcaagcactcaaaaagtgtgatggccaactcagcactgcacatgaggttgtgccctttgcagtgtttaagaactcaaagaaggtttatcttgataagcttgaccttaagactgaggagaatctgctaccagactcatttgtctgtttcgagcataagggacagtacaaaggaacaatggactctggtcagactaagagggagctcaaaagctttgatatctctcagtgccccaagattggaggacatggtagtaagaagtgcactggggacgcagcattttgctctgcttatgagtgcactgctcagtacgccaatgcctattgttcacatgctaatgggtcagggattgtgcagatacaagtatcaggggtctggaagaagcctttatgtgtagggtatgagagagtggttgtgaagagagaactctctgccaagcccatccagagagttgagccttgcacaacttgtataaccaaatgtgagcctcatggattggttgtccgatcaacagggttcaagatatcatcagcagttgcttgtgctagcggagtttgcgtcacaggatcgcagagtccttccaccgagattacactcaagtatccagggatatcccagtcttctgggggggacataggggttcacatggcacacgatgatcagtcagttagctccaaaatagtagctcactgccctccccaggacccgtgcttagtgcatgactgcatagtgtgtgctcatggcctgataaattaccagtgtcacactgctctcagtgcctttgttgttgtgtttgtattcagttctattgcaataatttgtttagctattctttatagggtgcttaagtgcctgaagattgccccaaggaaagttctgaatccactaatgtggatcacagccttcatcagatggatatataagaagatggttgccagagtggcagacaacattaatcaagtgaacagggaaataggatggatggaaggaggtcagttggttctagggaaccctgcccctattcctcgtcatgccccaatcccacgttatagcacatacctgatgttattattgattgtctcatatgcatcagcatgttcagaactgattcaggcaagctccagaatcaccacttgctctacagagggtgttaacaccaagtgtagactgtctggcacagcattgatcagagcagggtcagttggggcagaggcttgtttgatgttgaagggggtcaaggaagatcaaaccaagttcttaaagataaaaactgtctcaagtgagctatcatgcagggagggccagagttattggactgggtcctttagccctaaatgtttgagctcaaggagatgccaccttgtcggggaatgccatgtgaataggtgtctgtcttggagggacaatgaaacttcagcagagttttcatttgttggggaaagcacgaccatgcgagagaataagtgttttgagcaatgtggaggatgggggtgtgggtgtttcaatgtgaacccatcttgcttatttgtgcacacgtatctgcagtcagttagaaaagaggcccttagagtttttaactgtatcgactgggtgcataaactcactctagagatcacagactttgatggctctgtttcaacaatagacttgggagcatcatctagccgtttcacaaactggggttcagttagcctctcactggacgcagagggcatttcaggctcaaatagcttttctttcattgagagcccaggcaaagggtatgcaattgttgatgagccattctcagaaattcctcggcaagggttcttgggggagatcaggtgcaattcagagtcctcagtcctgagtgctcatgaatcatgccttagggcaccaaaccttatctcatacaagcccatgatagatcaattggagtgcacaacaaatctgattgatccctttgttgtctttgagaggggttctctgccacagacaaggaatgacaaaacctttgcagcttcaaaaggaaatagaggtgttcaagctttctctaagggctctgtacaagctgatctaactctgatgtttgacaattttgaggtggactttgtgggagcagccgtatcttgtgatgccgccttcttaaatttgacaggttgctattcttgcaatgcaggggccagggtctgcctgtctatcacatccacaggaactggatctctctctgcccacaataaggatgggtctctgcatatagtccttccatcagagaatggaacaaaagaccagtgtcagatactacacttcactgtgcctgaagtagaggaggagtttatgtactcttgtgatggagatgagcggcctctgttggtgaaggggaccctgatagccattgatccatttgatgataggcgggaagcagggggggaatcaacagttgtgaatccaaaatctggatcttggaatttctttgactggttttctggactcatgagttggtttggagggcctcttaaaactatactcctcatttgcctgtatgttgcattatcaattgggctctttttcctccttatatatcttggaagaacaggcctctctaaaatgtggcttgctgccactaagaaggcctcatagatcagtacgtgtaaaagcaatatgttgaaataagtagacataagcaaacctaattatgtaagtattgtacagataggtcaaattattggaatatccaagcttagaaacttatgcaataatactttagatgtaagcttagttgtaatttggggtggtggggtgaggcagcagcagtctcaagtgcttgtgaatattctagttggcgtaatcgtcttttgccagattagctgggaattaaactaactctttgaagttgcaccggtctttgtgt

SEQ ID NO: 53 - DNA, 1690 bp, Artificial Sequence
  ZH548 RVF virus S segment
  gene 35..832: /note="ZH548 RVF virus gene encoding NSs protein"
  gene 915..1652: /note="ZH548 RVF virus gene encoding N protein"
acacaaagaccccctagtgcttatcaagtatatcatggattactttcctgtgatatctgttgatttgcagagtggtcgtcgtgttgtgtcagtggagtactttagaggagatggtcctcccaggataccttattctatggttgggccctgttgtgtctttctcatgcaccatcgtcctagtcacgaggttcgcttgcgattctctgatttctacaatgtcggagaattcccataccgagtcggacttggagactttgcatcaaacgttgcacctccaccagcgaagccttttcagagacttattgatctaataggccatatgactcttagtgatttcacaaggttccccaatctgaaagaagccatatcctggcctcttggagaaccctcactggctttctttgacctaagctctactagagtgcataggaatgatgacattagaagggatcagattgccactctagcaatgaggagttgcaagatcaccaatgatctagaggactcctttgttggcttacacaggatgatagcgactgaggccatcctcagagggattgacctgtgcctgttgccaggctttgatctcatgtatgaggttgctcacgtacagtgcgttcggcttctgcaagcagcaaaagaggacatttctaatgctgtagttccaaactcagccctcattgttcttatggaggagagcctgatgctgcgctcatcacttcccagcatgatggggagaaacaactggattccagttattcctccaatcccagatgttgagatggaatcagaggaggagagtgatgatgatggatttgttgaggttgattagaggttaaggctgccccaccccccaccccccaatcccgaccgtaaccccaactccccttccccccaaccccctgggcagccacttaggctgctgtcttgtaagcctgagcggctgccatgacagcagctgacggcttcccattggaatccacaagtccaaaggctttcaagaattctctcctcttctcatggcttataaagttgctattcactgctgcattcattggctgcgtgaacgttgcagcaacctcctcttttgttctacctcggaggtttgggttgatgacccgggagaactgcagcagatacagagagtgagcatctaatattgcccttagatagtctcctggtagagaaggatccaccatgccagcaaagctggggtgcatcatatgcctcgggtatgcaggggataggccgtccatggtagtcccagtgacaggaagccactcactcaagacgaccaaagcctggcatgtccagccagccaaggcggcagcaactcgtgatagagtcaactcatcccgggaaggattcccttcctttagcttatacttgttgatgagagcctccacagttgctttgccttctttcgacattttcatcatcatcctcctgggcttgttgccacgagttagagccagaacaatcattttcttggcatccttctcccagtcagccccaccatactgctttaagagttcgataactctacgggcatcaaacccttgataagcaaactctcggacccactgttcaatctcattgcggtccactgcttgagcagcaaactggatcgcaagctcttgatagttgtccattattgtaatagtgtttgtatctctagggagctttgtgt

SEQ ID NO: 54 - protein, 2092 aa, Artificial Sequence
  ZH548 RVFV L protein
MDSILSKQLVDKTGFVRVPIKHFDCTMLTLALPTFDVSKMVDRITIDFNLDDIQGASEIGSTLLPSMSIDVEDMANFVHDFTFGHLADKTDRLLMREFPMMNDGFDHLSPDMIIKTTSGMYNIVEFTTFRGDERGAFQAAMTKLAKYEVPCENRSQGRTVVLYVVSAYRHGVWSNLELEDSEAEEMVYRYRLALSVMDELRTLFPELSSTDEELGKTERELLAMVSSIQINWSVTESVFPPFSREMFDRFRSSPPDSEYITRIVSRCLINSQEKLINSSFFAEGNDKALRFSKNAEECSLAVERALNQYRAEDNLRDLNDHKSTIQLPPWLSYHDVDGKDLCPLQGLDVRGDHPMCNLWREVVTSANLEEIERMHDDAAAELEFALSGVKDRPDERNRYHRVHLNMGSDDSVYIAALGVNGKKHKADTLVQQMRDRSKQPFSPDHDVDHISEFLSACSSDLWATDEDLYSPLSCDKELRLAAQRIHQPSLSERGFNEIITEHYKFMGSRIGSWCQMVSLIGAELSASVKQHVKPNYFVIKRLLGSGIFLLIKPTSSKSHIFVSFAIKRSCWAFDLSTSRVFKPYIDAGDLLVTDFVSYKLSKLTNLCKCVSLMESSFSFWAEAFGIPSWNFVGDLFRSSDSAAMDASYMGKLSLLTLLEDKAATEELQTIARYIIMEGFVSPPEIPKPHKMTSKFPKVLRSELQVYLLNCLCRTIQRIAGEPFILKKKDGSISWGGMFNPFSGRPLLDMQPLISCCYNGYFKNKEEETEPSSLSGMYKKIIELEHLRPQSDAFLGYKDPELPRMHEFSVSYLKEACNHAKLVLRSLYGQNFMEQIDNQIIRELSGLTLERLATLKATSNFNENWYVYKDVADKNYTRDKLLVKMSKYASEGKSLAIQKFEDCMRQIESQGCMHICLFKKQQHGGLREIYVMGAEERIVQSVVETIARSIGKFFASDTLCNPPNKVKIPETHGIRARKQCKGPVWTCATSDDARKWNQGHFVTKFALMLCEFTSPKWWPLIIRGCSMFTRKRMMMNLNYLKILDGHRELDIRDDFVMDLFKAYHGEAEVPWAFKGKTYLETTTGMMQGILHYTSSLLHTIHQEYIRSLSFKIFNLKVAPEMSKSLVCDMMQGSDDSSMLISFPADDEKVLTRCKVAAAICFRMKKELGVYLAIYPSEKSTANTDFVMEYNSEFYFHTQHVRPTIRWIAACCSLPEVETLVARQEEASNLMTSVTEGGGSFSLAAMIQQAQCTLHYMLMGMGVSELFLEYKKAVLKWNDPGLGFFLLDNPYACGLGGFRFNLFKAITRTDLQKLYAFFMKKVKGSAARDWADEDVTIPETCSVSPGGALILSSSLKWGSRKKFQKLRDRLNIPENWIELINENPEVLYRAPRTGPEILLRIAEKVHSPGVVSSLSSGNAVCKVMASAVYFLSATIFEDTGRPEFNFLEDSKYSLLQKMAAYSGFHGFNDMEPEDILFLFPNIEELESLDSIVYNKGEIDIIPRVNIRDATQTRVTIFNEQKTLRTSPEKLVSDKWFGTQKSRIGKTTFLAEWEKLKKIVKWLEDTPEATLAHTPLNNHIQVRNFFARMESKPRTVRITGAPVKKRSGVSKIAMVIRDNFSRMGHLRGVEDLAGFTRSVSAEILKHFLFCILQGPYSESYKLQLIYRVLSSVSNVEIKESDGKTKTNLIGILQRFLDGDHVVPIIEEMGAGTVGGFIKRQQSKVVQNKVVYYGVGIWRGFMDGYQVHLEIENDIGQPPRLRNVTTNCQSSPWDLSIPIRQWAEDMGVTNNQDYSSKSSRGARYWMHSFRMQGPSKPFGCPVYIIKGDMSDVIRLRKEEVEMKVRGSTLNLYTKHHSHQDLHILSYTASDNDLSPGIFKSISDEGVAQALQLFEREPSNCWVRCESVAPKFISAILEICEGKRQIKGINRTRLSEIVRICSESSLRSKVGSMFSFVANVEEAHDVDYDALMDLMIEDAKNNAFSHVVDCIELDVSGPYEMESFDTSDVNLFGPAHYKDISSLSMIAHPLMDKFVDYAISKMGRASVRKVLETGRCSSKDYDLSKVLFRTLQRPEESIRIDDLELYEETDVADDMLG

SEQ ID NO: 55 - protein, 1197 aa, Artificial Sequence
  ZH548 RVFV M (poly)protein
MYVLLTILISVLVCEAVIRVSLSSTREETCFGDSTNPEMIEGAWDSLREEEMPEELSCSISGIREVKTSSQELYRALKAIIAADGLNNITCHGKDPEDKISLIKGPPHKKRVGIVRCERRRDAKQIGRETMAGIAMTVLPALAVFALAPVVFAEDPHLRNRPGKGHNYIDGMTQEDATCKPVTYAGACSSFDVLLEKGKFPLFQSYAHHRTLLEAVHDTIIAKADPPSCDLLSAHGNPCMKEKLVMKTHCPNDYQSAHYLNNDGKMASVKCPPKYELTEDCNFCRQMTGASLKKGSYPLQDLFCQSSEDDGSKLKTKMKGVCEVGVQALKKCDGQLSTAHEVVPFAVFKNSKKVYLDKLDLKTEENLLPDSFVCFEHKGQYKGTMDSGQTKRELKSFDISQCPKIGGHGSKKCTGDAAFCSAYECTAQYANAYCSHANGSGIVQIQVSGVWKKPLCVGYERVVVKRELSAKPIQRVEPCTTCITKCEPHGLVVRSTGFKISSAVACASGVCVTGSQSPSTEITLKYPGISQSSGGDIGVHMAHDDQSVSSKIVAHCPPQDPCLVHDCIVCAHGLINYQCHTALSAFVVVFVFSSIAIICLAILYRVLKCLKIAPRKVLNPLMWITAFIRWIYKKMVARVADNINQVNREIGWMEGGQLVLGNPAPIPRHAPIPRYSTYLMLLLIVSYASACSELIQASSRITTCSTEGVNTKCRLSGTALIRAGSVGAEACLMLKGVKEDQTKFLKIKTVSSELSCREGQSYWTGSFSPKCLSSRRCHLVGECHVNRCLSWRDNETSAEFSFVGESTTMRENKCFEQCGGWGCGCFNVNPSCLFVHTYLQSVRKEALRVFNCIDWVHKLTLEITDFDGSVSTIDLGASSSRFTNWGSVSLSLDAEGISGSNSFSFIESPGKGYAIVDEPFSEIPRQGFLGEIRCNSESSVLSAHESCLRAPNLISYKPMIDQLECTTNLIDPFVVFERGSLPQTRNDKTFAASKGNRGVQAFSKGSVQADLTLMFDNFEVDFVGAAVSCDAAFLNLTGCYSCNAGARVCLSITSTGTGSLSAHNKDGSLHIVLPSENGTKDQCQILHFTVPEVEEEFMYSCDGDERPLLVKGTLIAIDPFDDRREAGGESTVVNPKSGSWNFFDWFSGLMSWFGGPLKTILLICLYVALSIGLFFLLIYLGRTGLSKMWLAATKKAS

SEQ ID NO: 56 - protein, 265 aa, Artificial Sequence
  ZH548 RVFV NSs protein
MDYFPVISVDLQSGRRVVSVEYFRGDGPPRIPYSMVGPCCVFLMHHRPSHEVRLRFSDFYNVGEFPYRVGLGDFASNVAPPPAKPFQRLIDLIGHMTLSDFTRFPNLKEAISWPLGEPSLAFFDLSSTRVHRNDDIRRDQIATLAMRSCKITNDLEDSFVGLHRMIATEAILRGIDLCLLPGFDLMYEVAHVQCVRLLQAAKEDISNAVVPNSALIVLMEESLMLRSSLPSMMGRNNWIPVIPPIPDVEMESEEESDDDGFVEVD

SEQ ID NO: 57 - protein, 245 aa, Artificial Sequence
  ZH548 RVFV N protein
MDNYQELAIQFAAQAVDRNEIEQWVREFAYQGFDARRVIELLKQYGGADWEKDAKKMIVLALTRGNKPRRMMMKMSKEGKATVEALINKYKLKEGNPSRDELTLSRVAAALAGWTCQALVVLSEWLPVTGTTMDGLSPAYPRHMMHPSFAGMVDPSLPGDYLRAILDAHSLYLLQFSRVINPNLRGRTKEEVAATFTQPMNAAVNSNFISHEKRREFLKAFGLVDSNGKPSAAVMAAAQAYKTAA